European Patent Application EP 4 230 222 A1, published August 23, 2023. Title: METHOD. Applicant: Oxsonics Limited ADC Therapeutics S.A. The sequence listing filed with the application follows.

SEQUENCE LISTING (13 sequences)

SEQ ID NO: 1 - protein, 122 aa, Mus musculus
QVQLVESGGGVVQPGRSLRLSCAASGFTFSSYGMSWVRQAPGKGLEWVATISSGGSYTYYPDSVKGRFTISRDNSKNTLYLQMNSLRAEDTAVYYCARHPIYYTYDDTMDYWGQGTTVTVSS

SEQ ID NO: 2 - protein, 108 aa, Mus musculus
EIVLTQSPGTLSLSPGERATLSCSASSSVSSGNFHWYQQKPGLAPRLLIYRTSNLASGIPARFSGSGSGTDFTLTISSLEPEDFAVYYCQQWSGYPWTFGGGTKLEIK

SEQ ID NO: 3 - protein, 10 aa, Mus musculus
GFTFSSYGMS

SEQ ID NO: 4 - protein, 26 aa, Mus musculus
TISSGGSYTYYPDSVKGRFTISRDNS

SEQ ID NO: 5 - protein, 13 aa, Mus musculus
HPIYYTYDDTMDY

SEQ ID NO: 6 - protein, 12 aa, Mus musculus
SASSSVSSGNFH

SEQ ID NO: 7 - protein, 7 aa, Mus musculus
RTSNLAS

SEQ ID NO: 8 - protein, 9 aa, Mus musculus
QQWSGYPWT

SEQ ID NO: 9 - protein, 451 aa, Mus musculus
QVQLVESGGGVVQPGRSLRLSCAASGFTFSSYGMSWVRQAPGKGLEWVATISSGGSYTYYPDSVKGRFTISRDNSKNTLYLQMNSLRAEDTAVYYCARHPIYYTYDDTMDYWGQGTTVTVSSASTKGPSVFPLAPSSKSTSGGTAALGCLVKDYFPEPVTVSWNSGALTSGVHTFPAVLQSSGLYSLSSVVTVPSSSLGTQTYICNVNHKPSNTKVDKKVEPKSCDKTHTCPPCPAPELLGGPSVFLFPPKPKDTLMISRTPEVTCVVVDVSHEDPEVKFNWYVDGVEVHNAKTKPREEQYNSTYRVVSVLTVLHQDWLNGKEYKCKVSNKALPAPIEKTISKAKGQPREPQVYTLPPSREEMTKNQVSLTCLVKGFYPSDIAVEWESNGQPENNYKTTPPVLDSDGSFFLYSKLTVDKSRWQQGNVFSCSVMHEALHNHYTQKSLSLSPG

SEQ ID NO: 10 - protein, 215 aa, Mus musculus
EIVLTQSPGTLSLSPGERATLSCSASSSVSSGNFHWYQQKPGLAPRLLIYRTSNLASGIPARFSGSGSGTDFTLTISSLEPEDFAVYYCQQWSGYPWTFGGGTKLEIKRTVAAPSVFIFPPSDEQLKSGTASVVCLLNNFYPREAKVQWKVDNALQSGNSQESVTEQDSKDSTYSLSSTLTLSKADYEKHKVYACEVTHQGLSSPVTKSFNRGEC

SEQ ID NO: 11 - protein, 894 aa, Homo sapiens
MAWRCPRMGRVPLAWCLALCGWACMAPRGTQAEESPFVGNPGNITGARGLTGTLRCQLQVQGEPPEVHWLRDGQILELADSTQTQVPLGEDEQDDWIVVSQLRITSLQLSDTGQYQCLVFLGHQTFVSQPGYVGLEGLPYFLEEPEDRTVAANTPFNLSCQAQGPPEPVDLLWLQDAVPLATAPGHGPQRSLHVPGLNKTSSFSCEAHNAKGVTTSRTATITVLPQQPRNLHLVSRQPTELEVAWTPGLSGIYPLTHCTLQAVLSDDGMGIQAGEPDPPEEPLTSQASVPPHQLRLGSLHPHTPYHIRVACTSSQGPSSWTHWLPVETPEGVPLGPPENISATRNGSQAFVHWQEPRAPLQGTLLGYRLAYQGQDTPEVLMDIGLRQEVTLELQGDGSVSNLTVCVAAYTAAGDGPWSLPVPLEAWRPGQAQPVHQLVKEPSTPAFSWPWWYVLLGAVVAAACVLILALFLVHRRKKETRYGEVFEPTVERGELVVRYRVRKSYSRRTTEATLNSLGISEELKEKLRDVMVDRHKVALGKTLGEGEFGAVMEGQLNQDDSILKVAVKTMKIAICTRSELEDFLSEAVCMKEFDHPNVMRLIGVCFQGSERESFPAPVVILPFMKHGDLHSFLLYSRLGDQPVYLPTQMLVKFMADIASGMEYLSTKRFIHRDLAARNCMLNENMSVCVADFGLSKKIYNGDYYRQGRIAKMPVKWIAIESLADRVYTSKSDVWSFGVTMWEIATRGQTPYPGVENSEIYDYLRRGNRLKQPADCLDGLYALMSRCWELNPQDRPSFTELREDLENTLKALPPAQEPDEILYVNMDEGGGYPEPPGAAGGADPPTQPDPKDSCSCLTAAEVHPAGRYVLCPSTTPSPAQPADRGSPAAPGQEDGA

SEQ ID NO: 12 - protein, 4 aa, Artificial Sequence
  tetrapeptide linker
GGFG

SEQ ID NO: 13 - protein, 4 aa, Artificial Sequence
  tetrapeptide linker
GFGG